European Patent Application EP 4 378 481 A1, published June 5, 2024. Title: Medicinal composition for the treatment of Pancreatic Adenocarcinoma and Cholangiocarcinoma. Applicant: Japan Science and Technology Agency. Application JP. The sequence listing filed with the application follows.

SEQUENCE LISTING (10 sequences)

SEQ ID NO: 1 - DNA, 21 bp, synthetic construct
  source 1..21: mol_type = other DNA
aacctcaagatccacaagcgt

SEQ ID NO: 2 - DNA, 20 bp, synthetic construct
  source 1..20: mol_type = other DNA
cactggtgtggacatgggaa

SEQ ID NO: 3 - DNA, 20 bp, synthetic construct
  source 1..20: mol_type = other DNA
agcctcccgcttcgctctct

SEQ ID NO: 4 - DNA, 20 bp, synthetic construct
  source 1..20: mol_type = other DNA
ccaggcgcccaatacgacca

SEQ ID NO: 5 - RNA, 19 nt, synthetic construct
  source 1..19: mol_type = other RNA
ggctgtgacaaatcctaca

SEQ ID NO: 6 - RNA, 21 nt, synthetic construct
  source 1..21: mol_type = other RNA
aagattcgaggctgtgacaaa

SEQ ID NO: 7 - RNA, 19 nt, synthetic construct
  source 1..19: mol_type = other RNA
atccgcgcgatagtacgta

SEQ ID NO: 8 - RNA, 21 nt, synthetic construct
  source 1..21: mol_type = other RNA
aattctccgaacgtgtcacgt

SEQ ID NO: 9 - RNA, 19 nt, synthetic construct
  source 1..19: mol_type = other RNA
ggctgtgacaaatcctaca

SEQ ID NO: 10 - RNA, 19 nt, synthetic construct
  source 1..19: mol_type = other RNA
gtgatgaatccagcctaca